European Patent Application EP 4 567 110 A1, published June 11, 2025. Title: METHOD FOR PRODUCING OLIGONUCLEOTIDE. Applicant: 味の素株式会社. The sequence listing filed with the application follows.

SEQUENCE LISTING (80 sequences)

SEQ ID NO: 1 - DNA, 20 bp, synthetic construct
  source 1..20: mol_type = other DNA; note = Product oligo
tcttggttacatgaaatccc

SEQ ID NO: 2 - DNA, 10 bp, synthetic construct
  source 1..10: mol_type = other DNA; note = 5'-terminal substrate oligo
tcttggttac

SEQ ID NO: 3 - DNA, 10 bp, synthetic construct
  source 1..10: mol_type = other DNA; note = 3'-terminal substrate oligo
atgaaatccc

SEQ ID NO: 4 - DNA, 18 bp, synthetic construct
  source 1..18: mol_type = other DNA; note = Perfect complementary oligo
ggatttcatgtaaccaag

SEQ ID NO: 5 - DNA, 18 bp, synthetic construct
  source 1..18: mol_type = other DNA; note = Complementary oligo
  modified_base 9: mod_base = OTHER; note = abasic site
ggatttcangtaaccaag

SEQ ID NO: 6 - DNA, 22 bp, synthetic construct
  source 1..22: mol_type = other DNA; note = Complementary oligo
  modified_base 13: mod_base = OTHER; note = abasic site
ggattaatttcangtaaccaag

SEQ ID NO: 7 - DNA, 22 bp, synthetic construct
  source 1..22: mol_type = other DNA; note = Complementary oligo
  modified_base 9: mod_base = OTHER; note = abasic site
ggatttcangtaaccggccaag

SEQ ID NO: 8 - DNA, 26 bp, synthetic construct
  source 1..26: mol_type = other DNA; note = Complementary oligo
  modified_base 13: mod_base = OTHER; note = abasic site
ggattaatttcangtaaccggccaag

SEQ ID NO: 9 - DNA, 26 bp, synthetic construct
  source 1..26: mol_type = other DNA; note = Complementary oligo
ggattaatttcatgtaaccggccaag

SEQ ID NO: 10 - DNA, 22 bp, synthetic construct
  source 1..22: mol_type = other DNA; note = Complementary oligo
ggattaatttcatgtaaccaag

SEQ ID NO: 11 - DNA, 22 bp, synthetic construct
  source 1..22: mol_type = other DNA; note = Complementary oligo
ggatttcatgtaaccggccaag

SEQ ID NO: 12 - DNA, 17 bp, synthetic construct
  source 1..17: mol_type = other DNA; note = Complementary oligo
ggattcatgtaaccaag

SEQ ID NO: 13 - DNA, 16 bp, synthetic construct
  source 1..16: mol_type = other DNA; note = Complementary oligo
ggatcatgtaaccaag

SEQ ID NO: 14 - DNA, 15 bp, synthetic construct
  source 1..15: mol_type = other DNA; note = Complementary oligo
ggacatgtaaccaag

SEQ ID NO: 15 - DNA, 17 bp, synthetic construct
  source 1..17: mol_type = other DNA; note = Complementary oligo
ggatttcatgtaacaag

SEQ ID NO: 16 - DNA, 16 bp, synthetic construct
  source 1..16: mol_type = other DNA; note = Complementary oligo
ggatttcatgtaaaag

SEQ ID NO: 17 - DNA, 15 bp, synthetic construct
  source 1..15: mol_type = other DNA; note = Complementary oligo
ggatttcatgtaaag

SEQ ID NO: 18 - DNA, 19 bp, synthetic construct
  source 1..19: mol_type = other DNA; note = Complementary oligo
ggattttcatgtaaccaag

SEQ ID NO: 19 - DNA, 20 bp, synthetic construct
  source 1..20: mol_type = other DNA; note = Complementary oligo
ggatatttcatgtaaccaag

SEQ ID NO: 20 - DNA, 21 bp, synthetic construct
  source 1..21: mol_type = other DNA; note = Complementary oligo
ggattatttcatgtaaccaag

SEQ ID NO: 21 - DNA, 23 bp, synthetic construct
  source 1..23: mol_type = other DNA; note = Complementary oligo
ggattgaatttcatgtaaccaag

SEQ ID NO: 22 - DNA, 24 bp, synthetic construct
  source 1..24: mol_type = other DNA; note = Complementary oligo
ggattgcaatttcatgtaaccaag

SEQ ID NO: 23 - DNA, 25 bp, synthetic construct
  source 1..25: mol_type = other DNA; note = Complementary oligo
ggattgccaatttcatgtaaccaag

SEQ ID NO: 24 - DNA, 26 bp, synthetic construct
  source 1..26: mol_type = other DNA; note = Complementary oligo
ggattgcgcaatttcatgtaaccaag

SEQ ID NO: 25 - DNA, 19 bp, synthetic construct
  source 1..19: mol_type = other DNA; note = Complementary oligo
ggatttcatgtaacccaag

SEQ ID NO: 26 - DNA, 20 bp, synthetic construct
  source 1..20: mol_type = other DNA; note = Complementary oligo
ggatttcatgtaaccgcaag

SEQ ID NO: 27 - DNA, 21 bp, synthetic construct
  source 1..21: mol_type = other DNA; note = Complementary oligo
ggatttcatgtaaccgccaag

SEQ ID NO: 28 - DNA, 23 bp, synthetic construct
  source 1..23: mol_type = other DNA; note = Complementary oligo
ggatttcatgtaaccggaccaag

SEQ ID NO: 29 - DNA, 24 bp, synthetic construct
  source 1..24: mol_type = other DNA; note = Complementary oligo
ggatttcatgtaaccggtaccaag

SEQ ID NO: 30 - DNA, 25 bp, synthetic construct
  source 1..25: mol_type = other DNA; note = Complementary oligo
ggatttcatgtaaccggtaaccaag

SEQ ID NO: 31 - DNA, 26 bp, synthetic construct
  source 1..26: mol_type = other DNA; note = Complementary oligo
ggatttcatgtaaccggttaaccaag

SEQ ID NO: 32 - DNA, 22 bp, synthetic construct
  source 1..22: mol_type = other DNA; note = Complementary oligo
ggatttaattcatgtaaccaag

SEQ ID NO: 33 - DNA, 22 bp, synthetic construct
  source 1..22: mol_type = other DNA; note = Complementary oligo
ggatttcgatcatgtaaccaag

SEQ ID NO: 34 - DNA, 22 bp, synthetic construct
  source 1..22: mol_type = other DNA; note = Complementary oligo
ggatttcatgcatgtaaccaag

SEQ ID NO: 35 - DNA, 22 bp, synthetic construct
  source 1..22: mol_type = other DNA; note = Complementary oligo
ggatttcatgtatataaccaag

SEQ ID NO: 36 - DNA, 22 bp, synthetic construct
  source 1..22: mol_type = other DNA; note = Complementary oligo
ggatttcatgtaattaaccaag

SEQ ID NO: 37 - DNA, 22 bp, synthetic construct
  source 1..22: mol_type = other DNA; note = Complementary oligo
ggatttcatgtaacgtaccaag

SEQ ID NO: 38 - DNA, 22 bp, synthetic construct
  source 1..22: mol_type = other DNA; note = Complementary oligo
ggatttcatgtaaccaaccaag

SEQ ID NO: 39 - DNA, 22 bp, synthetic construct
  source 1..22: mol_type = other DNA; note = Complementary oligo
ggatttcatgtaaccttccaag

SEQ ID NO: 40 - DNA, 22 bp, synthetic construct
  source 1..22: mol_type = other DNA; note = Complementary oligo
ggatttcatgtaaccccggaag

SEQ ID NO: 41 - DNA, 22 bp, synthetic construct
  source 1..22: mol_type = other DNA; note = Complementary oligo
ggatttcatgtaaggccccaag

SEQ ID NO: 42 - DNA, 22 bp, synthetic construct
  source 1..22: mol_type = other DNA; note = Complementary oligo
ggatttcatgtaaggaaccaag

SEQ ID NO: 43 - DNA, 22 bp, synthetic construct
  source 1..22: mol_type = other DNA; note = Complementary oligo
ggatttcatgtaaggttccaag

SEQ ID NO: 44 - DNA, 26 bp, synthetic construct
  source 1..26: mol_type = other DNA; note = Complementary oligo
ggattaatttcatgtatataaccaag

SEQ ID NO: 45 - DNA, 26 bp, synthetic construct
  source 1..26: mol_type = other DNA; note = Complementary oligo
ggatttcatgcatgtaaccggccaag

SEQ ID NO: 46 - DNA, 30 bp, synthetic construct
  source 1..30: mol_type = other DNA; note = Complementary oligo
ggattaatttcatgtatataaccatgcaag

SEQ ID NO: 47 - DNA, 30 bp, synthetic construct
  source 1..30: mol_type = other DNA; note = Complementary oligo
ggattaatttcatgtatataaccggccaag

SEQ ID NO: 48 - DNA, 30 bp, synthetic construct
  source 1..30: mol_type = other DNA; note = Complementary oligo
ggattaatttcatgcatgtaaccggccaag

SEQ ID NO: 49 - DNA, 34 bp, synthetic construct
  source 1..34: mol_type = other DNA; note = Complementary oligo
ggatatatttcatgcatgtatataaccggccaag

SEQ ID NO: 50 - DNA, 34 bp, synthetic construct
  source 1..34: mol_type = other DNA; note = Complementary oligo
ggattaatttcatgcatgtatataaccatgcaag

SEQ ID NO: 51 - DNA, 34 bp, synthetic construct
  source 1..34: mol_type = other DNA; note = Complementary oligo
ggattaatttcatgcatgtatataaccggccaag

SEQ ID NO: 52 - DNA, 34 bp, synthetic construct
  source 1..34: mol_type = other DNA; note = Complementary oligo
ggatatatttcatgcatgtatataaccatgcaag

SEQ ID NO: 53 - DNA, 18 bp, synthetic construct
  source 1..18: mol_type = other DNA; note = Complementary oligo
  modified_base 9: mod_base = OTHER; note = abasic site
  modified_base 14: mod_base = OTHER; note = abasic site
ggatttcangtaancaag

SEQ ID NO: 54 - DNA, 18 bp, synthetic construct
  source 1..18: mol_type = other DNA; note = Complementary oligo
  modified_base 4: mod_base = OTHER; note = abasic site
  modified_base 9: mod_base = OTHER; note = abasic site
gganttcangtaaccaag

SEQ ID NO: 55 - DNA, 18 bp, synthetic construct
  source 1..18: mol_type = other DNA; note = Complementary oligo
  modified_base 4: mod_base = OTHER; note = abasic site
  modified_base 9: mod_base = OTHER; note = abasic site
  modified_base 14: mod_base = OTHER; note = abasic site
gganttcangtaancaag

SEQ ID NO: 56 - DNA, 18 bp, synthetic construct
  source 1..18: mol_type = other DNA; note = Complementary oligo
ggatttcaagtaaccaag

SEQ ID NO: 57 - DNA, 18 bp, synthetic construct
  source 1..18: mol_type = other DNA; note = Complementary oligo
ggatttcaggtaaccaag

SEQ ID NO: 58 - DNA, 18 bp, synthetic construct
  source 1..18: mol_type = other DNA; note = Complementary oligo
ggatttcacgtaaccaag

SEQ ID NO: 59 - DNA, 18 bp, synthetic construct
  source 1..18: mol_type = other DNA; note = Complementary oligo
ggatttcatataaccaag

SEQ ID NO: 60 - DNA, 18 bp, synthetic construct
  source 1..18: mol_type = other DNA; note = Complementary oligo
ggatttcatttaaccaag

SEQ ID NO: 61 - DNA, 18 bp, synthetic construct
  source 1..18: mol_type = other DNA; note = Complementary oligo
ggatttcatctaaccaag

SEQ ID NO: 62 - DNA, 50 bp, synthetic construct
  source 1..50: mol_type = other DNA; note = 5'-terminal substrate oligo
ctggcataagcgtagcagtcctggcataagcgtagcagtctcttggttac

SEQ ID NO: 63 - DNA, 50 bp, synthetic construct
  source 1..50: mol_type = other DNA; note = 3'-terminal substrate oligo
atgaaatcccctggcataagcgtagcagtcctggcataagcgtagcagtc

SEQ ID NO: 64 - DNA, 50 bp, synthetic construct; identical to SEQ ID NO: 62
  source 1..50: mol_type = other DNA; note = 5'-terminal substrate oligo
  modified_base 2: mod_base = OTHER; note = 2'-O-methoxyethyl-thymidine
  modified_base 4: mod_base = OTHER; note = phosphorothioate DNA
  modified_base 6: mod_base = OTHER; note = 2'-O-methyl-deoxyadenosine
  modified_base 12: mod_base = OTHER; note = 2'-fluoro-deoxyguanosine
  modified_base 17: mod_base = OTHER; note = 2'-O-methoxyethyl-deoxyadenosine
  modified_base 20: mod_base = OTHER; note = phosphorothioate DNA
  modified_base 22: mod_base = OTHER; note = 2'-O-methyl-thymidine
  modified_base 29: mod_base = OTHER; note = 2'-fluoro-deoxyadenosine
  modified_base 33: mod_base = OTHER; note = phosphorothioate DNA
  modified_base 34: mod_base = OTHER; note = 2'-O-methoxyethyl-deoxyadenosine
  modified_base 41: mod_base = OTHER; note = 2'-fluoro-deoxyuridine
  modified_base 42: mod_base = OTHER; note = 2'-O-methyl-deoxycytidine
  modified_base 43: mod_base = OTHER; note = 2'-fluoro-deoxyuridine
  modified_base 44: mod_base = OTHER; note = 2'-O-methoxyethyl-thymidine
  modified_base 45: mod_base = OTHER; note = 2'-O-methoxyethyl-deoxyguanosine

SEQ ID NO: 65 - DNA, 50 bp, synthetic construct; identical to SEQ ID NO: 63
  source 1..50: mol_type = other DNA; note = 3'-terminal substrate oligo
  modified_base 6: mod_base = OTHER; note = 2'-O-methoxyethyl-deoxyadenosine
  modified_base 7: mod_base = OTHER; note = 2'-O-methoxyethyl-thymidine
  modified_base 8: mod_base = OTHER; note = 2'-fluoro-deoxycytidine
  modified_base 9: mod_base = OTHER; note = 2'-O-methyl-deoxycytidine
  modified_base 10: mod_base = OTHER; note = 2'-fluoro-deoxycytidine
  modified_base 15: mod_base = OTHER; note = phosphorothioate DNA
  modified_base 17: mod_base = OTHER; note = 2'-O-methoxyethyl-thymidine
  modified_base 21: mod_base = OTHER; note = 2'-O-methoxyethyl-5-methyldeoxycytidine
  modified_base 25: mod_base = OTHER; note = phosphorothioate DNA
  modified_base 28: mod_base = OTHER; note = 2'-O-methoxyethyl-deoxyguanosine
  modified_base 31: mod_base = OTHER; note = 2'-O-methoxyethyl-5-methyldeoxycytidine
  modified_base 34: mod_base = OTHER; note = 2'-O-methoxyethyl-deoxyguanosine
  modified_base 38: mod_base = OTHER; note = 2'-O-methoxyethyl-deoxyadenosine
  modified_base 42: mod_base = OTHER; note = phosphorothioate DNA
  modified_base 46: mod_base = OTHER; note = 2'-O-methoxyethyl-5-methyldeoxycytidine

SEQ ID NO: 66 - DNA, 20 bp, synthetic construct
  source 1..20: mol_type = other DNA; note = internal substrate oligo
atgaaatcccgcctcagtct

SEQ ID NO: 67 - DNA, 10 bp, synthetic construct
  source 1..10: mol_type = other DNA; note = 3'-terminal substrate oligo
gcttcgcacc

SEQ ID NO: 68 - DNA, 20 bp, synthetic construct
  source 1..20: mol_type = other DNA; note = Complementary oligo
ggtgcgaagcagactgaggc

SEQ ID NO: 69 - DNA, 16 bp, synthetic construct
  source 1..16: mol_type = other DNA; note = Complementary oligo
tgcgaagccgactgag

SEQ ID NO: 70 - DNA, 10 bp, synthetic construct
  source 1..10: mol_type = other DNA; note = 5'-terminal substrate oligo
  modified_base 1: mod_base = OTHER; note = 2'-O-methoxyethyl-thymidine
  modified_base 2: mod_base = OTHER; note = 2'-O-methyl-deoxycytidine (phosphorothioate DNA)
  modified_base 3: mod_base = OTHER; note = 2'-O-methoxyethyl-thymidine
  modified_base 4: mod_base = OTHER; note = 2'-O-methoxyethyl-thymidine
  modified_base 5: mod_base = OTHER; note = 2'-fluoro-deoxyguanosine
tcttggttac

SEQ ID NO: 71 - DNA, 20 bp, synthetic construct
  source 1..20: mol_type = other DNA; note = internal substrate oligo
  modified_base 6: mod_base = OTHER; note = 2'-O-methoxyethyl-deoxyadenosine
  modified_base 7: mod_base = OTHER; note = 2'-O-methoxyethyl-thymidine
  modified_base 8: mod_base = OTHER; note = 2'-fluoro-deoxycytidine
  modified_base 9: mod_base = OTHER; note = 2'-O-methoxyethyl-5-methyldeoxycytidine
  modified_base 10: mod_base = OTHER; note = 2'-O-methyl-deoxycytidine
  modified_base 11: mod_base = OTHER; note = 2'-O-methoxyethyl-deoxyguanosine
  modified_base 12: mod_base = OTHER; note = 2'-fluoro-deoxycytidine
  modified_base 13: mod_base = OTHER; note = 2'-O-methoxyethyl-5-methyldeoxycytidine
  modified_base 14: mod_base = OTHER; note = 2'-O-methoxyethyl-thymidine
  modified_base 15: mod_base = OTHER; note = 2'-O-methoxyethyl-5-methyldeoxycytidine
atgaaatcccgcctcagtct

SEQ ID NO: 72 - DNA, 10 bp, synthetic construct
  source 1..10: mol_type = other DNA; note = 3'-terminal substrate oligo
  modified_base 6: mod_base = OTHER; note = 2'-O-methoxyethyl-deoxyguanosine
  modified_base 7: mod_base = OTHER; note = 2'-O-methoxyethyl-5-methyldeoxycytidine
  modified_base 8: mod_base = OTHER; note = 2'-fluoro-deoxyadenosine
  modified_base 9: mod_base = OTHER; note = 2'-O-methyl-deoxycytidine (phosphorothioate DNA)
  modified_base 10: mod_base = OTHER; note = 2'-O-methoxyethyl-5-methyldeoxycytidine
gcttcgcacc

SEQ ID NO: 73 - DNA, 10 bp, synthetic construct
  source 1..10: mol_type = other DNA; note = 5'-terminal substrate oligo
  misc_feature 1..5: note = DNA
  misc_feature 6..10: note = RNA
  modified_base 1: mod_base = OTHER; note = 2'-O-methyl-deoxyuridine
  modified_base 2: mod_base = OTHER; note = 2'-O-methyl-deoxycytidine
  modified_base 3: mod_base = OTHER; note = 2'-O-methyl-deoxyuridine
  modified_base 4: mod_base = OTHER; note = 2'-O-methyl-deoxyuridine
  modified_base 5: mod_base = OTHER; note = 2'-O-methyl-deoxyguanosine
tcttggttac

SEQ ID NO: 74 - DNA, 10 bp, synthetic construct
  source 1..10: mol_type = other DNA; note = 3'-terminal substrate oligo
  misc_feature 1..5: note = RNA
  misc_feature 6..10: note = DNA
  modified_base 6: mod_base = OTHER; note = 2'-O-methyl-deoxyadenosine
  modified_base 7: mod_base = OTHER; note = 2'-O-methyl-deoxyuridine
  modified_base 8: mod_base = OTHER; note = 2'-O-methyl-deoxycytidine
  modified_base 9: mod_base = OTHER; note = 2'-O-methyl-deoxycytidine
  modified_base 10: mod_base = OTHER; note = 2'-O-methyl-deoxycytidine
atgaaatccc

SEQ ID NO: 75 - DNA, 10 bp, synthetic construct
  source 1..10: mol_type = other DNA; note = 5'-terminal substrate oligo
  modified_base 3: mod_base = OTHER; note = 2'-O-methoxyethyl-thymidine
tcttggttac

SEQ ID NO: 76 - DNA, 10 bp, synthetic construct
  source 1..10: mol_type = other DNA; note = 3'-terminal substrate oligo
  modified_base 8: mod_base = OTHER; note = 2'-O-methoxyethyl-deoxycytidine
atgaaatccc

SEQ ID NO: 77 - DNA, 10 bp, synthetic construct
  source 1..10: mol_type = other DNA; note = 5'-terminal substrate oligo
  modified_base 1: mod_base = OTHER; note = 2'-O-methoxyethyl-thymidine
  modified_base 2: mod_base = OTHER; note = 2'-O-methoxyethyl-deoxycytidine
  modified_base 3: mod_base = OTHER; note = 2'-O-methoxyethyl-thymidine
  modified_base 4: mod_base = OTHER; note = 2'-O-methoxyethyl-thymidine
  modified_base 5: mod_base = OTHER; note = 2'-O-methoxyethyl-deoxyguanosine
tcttggttac

SEQ ID NO: 78 - DNA, 10 bp, synthetic construct
  source 1..10: mol_type = other DNA; note = 3'-terminal substrate oligo
  modified_base 6: mod_base = OTHER; note = 2'-O-methoxyethyl-deoxyadenosine
  modified_base 7: mod_base = OTHER; note = 2'-O-methoxyethyl-thymidine
  modified_base 8: mod_base = OTHER; note = 2'-O-methoxyethyl-deoxycytidine
  modified_base 9: mod_base = OTHER; note = 2'-O-methoxyethyl-deoxycytidine
  modified_base 10: mod_base = OTHER; note = 2'-O-methoxyethyl-deoxycytidine
atgaaatccc

SEQ ID NO: 79 - DNA, 10 bp, synthetic construct
  source 1..10: mol_type = other DNA; note = 5'-terminal substrate oligo
  modified_base 2..10: mod_base = OTHER; note = phosphorothioate DNAs
tcttggttac

SEQ ID NO: 80 - DNA, 10 bp, synthetic construct
  source 1..10: mol_type = other DNA; note = 3'-terminal substrate oligo
  modified_base 2..10: mod_base = OTHER; note = phosphorothioate DNAs
atgaaatccc